European Patent Specification EP 3 740 565 B1, published June 10, 2026. Title: Generation, proliferation and expansion of epithelial cells from primary tissue into mucosoid cultures. Applicant: Max-Planck-Gesellschaft zur Förderung der Wissenschaft e.V. The sequence listing filed with the application follows.

SEQUENCE LISTING (76 sequences)

SEQ ID NO: 1 - DNA, 20 bp, Artificial Sequence
  CXCL1-3 Forward Primer
cgcccaaaccgaagtcatag

SEQ ID NO: 2 - DNA, 23 bp, Artificial Sequence
  CXCL1-3 Reverse Primer
gctccccttgttcagtatctttt

SEQ ID NO: 3 - DNA, 21 bp, Artificial Sequence
  CCL20 Forward Primer
tgctgtaccaagagtttgctc

SEQ ID NO: 4 - DNA, 23 bp, Artificial Sequence
  CCL20 Reverse Primer
cgcacacagacaactttttcttt

SEQ ID NO: 5 - DNA, 20 bp, Artificial Sequence
  LTB Forward Primer
gtacgggcctctctggtaca

SEQ ID NO: 6 - DNA, 20 bp, Artificial Sequence
  LTB Reverse Primer
gtccaccatatcggggtgac

SEQ ID NO: 7 - DNA, 21 bp, Artificial Sequence
  IL23A Forward Primer
ctcagggacaacagtcagttc

SEQ ID NO: 8 - DNA, 19 bp, Artificial Sequence
  IL23A Reverse Primer
acagggctatcagggagca

SEQ ID NO: 9 - DNA, 21 bp, Artificial Sequence
  KRT19 Forward Primer
gtcacagctgagcatgaaagc

SEQ ID NO: 10 - DNA, 19 bp, Artificial Sequence
  KRT19 Reverse Primer
agctgggcttcaataccgc

SEQ ID NO: 11 - DNA, 21 bp, Artificial Sequence
  KRT18 Forward Primer
ttctgggggcatgagcttcac

SEQ ID NO: 12 - DNA, 18 bp, Artificial Sequence
  KRT18 Reverse Primer
gcgcctgcatagacgctg

SEQ ID NO: 13 - DNA, 20 bp, Artificial Sequence
  KRT8 Forward Primer
gctggccgtaaactgctttg

SEQ ID NO: 14 - DNA, 20 bp, Artificial Sequence
  KRT8 Reverse Primer
acatttggcagccagctttg

SEQ ID NO: 15 - DNA, 20 bp, Artificial Sequence
  EPCAM Forward Primer
gctggccgtaaactgctttg

SEQ ID NO: 16 - DNA, 20 bp, Artificial Sequence
  EPCAM Reverse Primer
acatttggcagccagctttg

SEQ ID NO: 17 - DNA, 20 bp, Artificial Sequence
  CDH1 Forward Primer
taccctggtggttcaagctg

SEQ ID NO: 18 - DNA, 20 bp, Artificial Sequence
  CDH1 Reverse Primer
cctgacccttgtacgtggtg

SEQ ID NO: 19 - DNA, 20 bp, Artificial Sequence
  LGR5 Forward Primer
ctcccaggtctggtgtgttg

SEQ ID NO: 20 - DNA, 20 bp, Artificial Sequence
  LGR5 Reverse Primer
gctcgcaatgacagtgtgtg

SEQ ID NO: 21 - DNA, 20 bp, Artificial Sequence
  CTNNB Forward Primer
agcaatttgtggagggggtc

SEQ ID NO: 22 - DNA, 20 bp, Artificial Sequence
  CTNNB Reverse Primer
agcagctgcacaaacaatgg

SEQ ID NO: 23 - DNA, 20 bp, Artificial Sequence
  CD44 Forward Primer
agcaccatttcaaccacacc

SEQ ID NO: 24 - DNA, 20 bp, Artificial Sequence
  CD44 Reverse Primer
gcagtggtgccatttctgtc

SEQ ID NO: 25 - DNA, 21 bp, Artificial Sequence
  PGC Forward Primer
tgtctttgggggtgtggatag

SEQ ID NO: 26 - DNA, 24 bp, Artificial Sequence
  PGC Reverse Primer
atgaggaactcttcaatgccaatc

SEQ ID NO: 27 - DNA, 20 bp, Artificial Sequence
  MUC6 Forward Primer
cagctcaacaaggtgtgtgc

SEQ ID NO: 28 - DNA, 20 bp, Artificial Sequence
  MUC6 Reverse Primer
tggggaaaggtctcctcgta

SEQ ID NO: 29 - DNA, 20 bp, Artificial Sequence
  MUC5AC Forward Primer
ggaggtgcccacttctcaac

SEQ ID NO: 30 - DNA, 19 bp, Artificial Sequence
  MUC5AC Reverse Primer
cttcaggcaggtctcgctg

SEQ ID NO: 31 - DNA, 20 bp, Artificial Sequence
  CHGA Forward Primer
ccaaggagagggcacatcag

SEQ ID NO: 32 - DNA, 20 bp, Artificial Sequence
  CHGA Reverse Primer
tcttccaccgcctctttcag

SEQ ID NO: 33 - DNA, 20 bp, Artificial Sequence
  ATP4b Forward Primer
tgggtgtggatcagcctgta

SEQ ID NO: 34 - DNA, 20 bp, Artificial Sequence
  ATP4b Reverse Primer
ctggtcttggtagtccggtg

SEQ ID NO: 35 - DNA, 21 bp, Artificial Sequence
  IL-8 Forward Primer
acactgcgccaacacagaaat

SEQ ID NO: 36 - DNA, 21 bp, Artificial Sequence
  IL-8 Reverse Primer
attgcatctggcaaccctaca

SEQ ID NO: 37 - DNA, 20 bp, Artificial Sequence
  TNF Forward Primer
tccccagggacctctctcta

SEQ ID NO: 38 - DNA, 21 bp, Artificial Sequence
  TNF Reverse Primer
gagggtttgctacaacatggg

SEQ ID NO: 39 - DNA, 21 bp, Artificial Sequence
  sFRP1 Forward Primer
acgtgggctacaagaagatgg

SEQ ID NO: 40 - DNA, 19 bp, Artificial Sequence
  sFRP1 Reverse Primer
cagcgacacgggtagatgg

SEQ ID NO: 41 - DNA, 21 bp, Artificial Sequence
  sFRP2 Forward Primer 1
acgtgggctacaagaagatgg

SEQ ID NO: 42 - DNA, 19 bp, Artificial Sequence
  sFRP2 Reverse Primer 1
cagcgacacgggtagatgg

SEQ ID NO: 43 - DNA, 19 bp, Artificial Sequence
  sFRP2 Forward Primer 2
ctggcccgacatgcttgag

SEQ ID NO: 44 - DNA, 22 bp, Artificial Sequence
  sFRP2 Reverse Primer 2
gcttcacatacctttggagctt

SEQ ID NO: 45 - DNA, 22 bp, Artificial Sequence
  sFRP3 Forward Primer 2
acacagacttacagggcttgat

SEQ ID NO: 46 - DNA, 23 bp, Artificial Sequence
  sFRP3 Reverse Primer 2
gagcccatactcatcaagtaccg

SEQ ID NO: 47 - DNA, 19 bp, Artificial Sequence
  sFRP4 Forward Primer
cctggaacatcacgcggat

SEQ ID NO: 48 - DNA, 19 bp, Artificial Sequence
  sFRP4 Reverse Primer
cggcttgatagggtcgtgc

SEQ ID NO: 49 - DNA, 22 bp, Artificial Sequence
  sFRP5 Forward Primer
aggagtacgactactatggctg

SEQ ID NO: 50 - DNA, 19 bp, Artificial Sequence
  sFRP5 Reverse Primer
ggtcggcagggatgtcaag

SEQ ID NO: 51 - DNA, 23 bp, Artificial Sequence
  DKK1 Forward Primer
ccttgaactcggttctcaattcc

SEQ ID NO: 52 - DNA, 23 bp, Artificial Sequence
  DKK1 Reverse Primer
caatggtctggtacttattcccg

SEQ ID NO: 53 - DNA, 19 bp, Artificial Sequence
  DKK2 Forward Primer
ctcacagatcggcagttcg

SEQ ID NO: 54 - DNA, 21 bp, Artificial Sequence
  DKK2 Reverse Primer
atgccagtccttggtacatgc

SEQ ID NO: 55 - DNA, 20 bp, Artificial Sequence
  DKK3 Forward Primer 1
aggacacgcagcacaaattg

SEQ ID NO: 56 - DNA, 23 bp, Artificial Sequence
  DKK3 Reverse Primer 1
ccagtctggttgttggttatctt

SEQ ID NO: 57 - DNA, 20 bp, Artificial Sequence
  DKK3 Forward Primer 2
acgagtgcatcatcgacgag

SEQ ID NO: 58 - DNA, 20 bp, Artificial Sequence
  DKK3 Reverse Primer 2
gcagtccctctggttgtcac

SEQ ID NO: 59 - DNA, 21 bp, Artificial Sequence
  DKK4 Forward Primer
acggactgcaataccagaaag

SEQ ID NO: 60 - DNA, 21 bp, Artificial Sequence
  DKK4 Reverse Primer
cgttcacacagagtgtcccag

SEQ ID NO: 61 - DNA, 21 bp, Artificial Sequence
  DKKL1 Forward Primer
ctctaccctggtgatcccctc

SEQ ID NO: 62 - DNA, 22 bp, Artificial Sequence
  DKKL1 Reverse Primer
cgaagcaggttacctttcagga

SEQ ID NO: 63 - DNA, 23 bp, Artificial Sequence
  USAG1 Forward Primer
gccatcagagatgtatttggtgg

SEQ ID NO: 64 - DNA, 21 bp, Artificial Sequence
  USAG1 Reverse Primer
gtgctccctaactggattgga

SEQ ID NO: 65 - DNA, 22 bp, Artificial Sequence
  WIF1 Forward Primer
tctccaaacacctcaaaatgct

SEQ ID NO: 66 - DNA, 19 bp, Artificial Sequence
  WIF1 Reverse Primer
gacactcgcagatgcgtct

SEQ ID NO: 67 - DNA, 21 bp, Artificial Sequence
  BARX1 Forward Primer
ttccacgccggacagaataga

SEQ ID NO: 68 - DNA, 20 bp, Artificial Sequence
  BARX1 Reverse Primer
agtaagctgctcgctcgttg

SEQ ID NO: 69 - DNA, 19 bp, Artificial Sequence
  TFF2 Forward Primer
cggggagtgagaaaccctc

SEQ ID NO: 70 - DNA, 21 bp, Artificial Sequence
  TFF2 Reverse Primer
cactggagtcgaaacagcatc

SEQ ID NO: 71 - DNA, 23 bp, Artificial Sequence
  GAPDH Forward Primer
ggtatcgtggaaggactcatgac

SEQ ID NO: 72 - DNA, 23 bp, Artificial Sequence
  GAPDH Reverse Primer
atgccagtgagcttcccgttcag

SEQ ID NO: 73 - DNA, 31 bp, Artificial Sequence
  rDNA 16s H.pylori Forward Primer
tttgttagagaagataatgacggtatctaac

SEQ ID NO: 74 - DNA, 28 bp, Artificial Sequence
  rDNA 16s H.pylori Reverse Primer
cataggatttcacacctgactgactatc

SEQ ID NO: 75 - DNA, 19 bp, Artificial Sequence
  gDNA hGAPDH Forward Primer
gacttcaacagcgacaccc

SEQ ID NO: 76 - DNA, 25 bp, Artificial Sequence
  gDNA hGAPDH Reverse Primer
agaagatgaaaagagttgtcagggc